European Patent Specification EP 3 319 983 B1, published January 28, 2026. Title: Tau-binding antibodies. Applicant: UCB BIOPHARMA sprl. The sequence listing filed with the application follows.

SEQUENCE LISTING (57 sequences)

SEQ ID NO: 1 - protein, 16 aa, Rattus norvegicus
RSSQSLEYSDGYTYLE

SEQ ID NO: 2 - protein, 7 aa, Rattus norvegicus
EVSNRFS

SEQ ID NO: 3 - protein, 9 aa, Rattus norvegicus
FQATHNPYT

SEQ ID NO: 4 - protein, 10 aa, Rattus norvegicus
GFSLTSNDIA

SEQ ID NO: 5 - protein, 16 aa, Rattus norvegicus
  misc_feature (12)..(12): Xaa can be Ser, Ala, Thr
TIWTDGSTNYNXAVQS

SEQ ID NO: 6 - protein, 10 aa, Rattus norvegicus
HRLYYGAFDY

SEQ ID NO: 7 - protein, 112 aa, Rattus norvegicus
DIVMTQTPVSLSVTLGDQASISCRSSQSLEYSDGYTYLEWYLQKPGQSPQLLIYEVSNRFSGVPDRFIGSGSGTDFTLKISRVEPEDLGVYYCFQATHNPYTFGAGTKLEIK

SEQ ID NO: 8 - protein, 117 aa, Rattus norvegicus
EVKLEESGPGLMQPSETLSLTCTVSGFSLTSNDIAWVRQPLGKGLVWMGTIWTDGSTNYNSAVQSRLSISRDTSKSQFFLKMNSLQPEDTGTYYCARHRLYYGAFDYWGQGTMVTVS

SEQ ID NO: 9 - protein, 112 aa, Artificial Sequence
  humanized
DIVMTQTPLSLSVTPGQPASISCRSSQSLEYSDGYTYLEWYLQKPGQSPQLLIYEVSNRFSGVPDRFSGSGSGTDFTLKISRVEAEDVGVYYCFQATHNPYTFGQGTKLEIK

SEQ ID NO: 10 - protein, 118 aa, Artificial Sequence
  humanized
  MISC_FEATURE (48)..(48): Xaa can be Ile and Met
  MISC_FEATURE (61)..(61): Xaa can be Ser, Ala, Thr
ZVQLQESGPGLVKPSETLSLTCTVSGFSLTSNDIAWIRQPPGKGLEWXGTIWTDGSTNYNXAVQSRVTISVDTSKNQFSLKLSSVTAADTAVYYCARHRLYYGAFDYWGQGTMVTVSS

SEQ ID NO: 11 - protein, 118 aa, Artificial Sequence
  humanized
EVQLQESGPGLVKPSETLSLTCTVSGFSLTSNDIAWIRQPPGKGLEWMGTIWTDGSTNYNSAVQSRVTISVDTSKNQFSLKLSSVTAADTAVYYCARHRLYYGAFDYWGQGTMVTVSS

SEQ ID NO: 12 - protein, 118 aa, Artificial Sequence
  humanized
EVQLQESGPGLVKPSETLSLTCTVSGFSLTSNDIAWIRQPPGKGLEWMGTIWTDGSTNYNAAVQSRVTISVDTSKNQFSLKLSSVTAADTAVYYCARHRLYYGAFDYWGQGTMVTVSS

SEQ ID NO: 13 - protein, 118 aa, Artificial Sequence
  humanized
EVQLQESGPGLVKPSETLSLTCTVSGFSLTSNDIAWIRQPPGKGLEWMGTIWTDGSTNYNTAVQSRVTISVDTSKNQFSLKLSSVTAADTAVYYCARHRLYYGAFDYWGQGTMVTVSS

SEQ ID NO: 14 - protein, 219 aa, Artificial Sequence
  humanized
DIVMTQTPLSLSVTPGQPASISCRSSQSLEYSDGYTYLEWYLQKPGQSPQLLIYEVSNRFSGVPDRFSGSGSGTDFTLKISRVEAEDVGVYYCFQATHNPYTFGQGTKLEIKRTVAAPSVFIFPPSDEQLKSGTASVVCLLNNFYPREAKVQWKVDNALQSGNSQESVTEQDSKDSTYSLSSTLTLSKADYEKHKVYACEVTHQGLSSPVTKSFNRGEC

SEQ ID NO: 15 - protein, 445 aa, Artificial Sequence
  humanized
  misc_feature (48)..(48): Xaa can be Ile or Met
  misc_feature (61)..(61): Xaa can be Ser Ala or Thr
ZVQLQESGPGLVKPSETLSLTCTVSGFSLTSNDIAWIRQPPGKGLEWXGTIWTDGSTNYNXAVQSRVTISVDTSKNQFSLKLSSVTAADTAVYYCARHRLYYGAFDYWGQGTMVTVSSASTKGPSVFPLAPCSRSTSESTAALGCLVKDYFPEPVTVSWNSGALTSGVHTFPAVLQSSGLYSLSSVVTVPSSSLGTKTYTCNVDHKPSNTKVDKRVESKYGPPCPPCPAPEFLGGPSVFLFPPKPKDTLMISRTPEVTCVVVDVSQEDPEVQFNWYVDGVEVHNAKTKPREEQFNSTYRVVSVLTVLHQDWLNGKEYKCKVSNKGLPSSIEKTISKAKGQPREPQVYTLPPSQEEMTKNQVSLTCLVKGFYPSDIAVEWESNGQPENNYKTTPPVLDSDGSFFLYSRLTVDKSRWQEGNVFSCSVMHEALHNHYTQKSLSLSLGK

SEQ ID NO: 16 - protein, 445 aa, Artificial Sequence
  humanized
EVQLQESGPGLVKPSETLSLTCTVSGFSLTSNDIAWIRQPPGKGLEWMGTIWTDGSTNYNSAVQSRVTISVDTSKNQFSLKLSSVTAADTAVYYCARHRLYYGAFDYWGQGTMVTVSSASTKGPSVFPLAPCSRSTSESTAALGCLVKDYFPEPVTVSWNSGALTSGVHTFPAVLQSSGLYSLSSVVTVPSSSLGTKTYTCNVDHKPSNTKVDKRVESKYGPPCPPCPAPEFLGGPSVFLFPPKPKDTLMISRTPEVTCVVVDVSQEDPEVQFNWYVDGVEVHNAKTKPREEQFNSTYRVVSVLTVLHQDWLNGKEYKCKVSNKGLPSSIEKTISKAKGQPREPQVYTLPPSQEEMTKNQVSLTCLVKGFYPSDIAVEWESNGQPENNYKTTPPVLDSDGSFFLYSRLTVDKSRWQEGNVFSCSVMHEALHNHYTQKSLSLSLGK

SEQ ID NO: 17 - protein, 445 aa, Artificial Sequence
  humanized
EVQLQESGPGLVKPSETLSLTCTVSGFSLTSNDIAWIRQPPGKGLEWMGTIWTDGSTNYNAAVQSRVTISVDTSKNQFSLKLSSVTAADTAVYYCARHRLYYGAFDYWGQGTMVTVSSASTKGPSVFPLAPCSRSTSESTAALGCLVKDYFPEPVTVSWNSGALTSGVHTFPAVLQSSGLYSLSSVVTVPSSSLGTKTYTCNVDHKPSNTKVDKRVESKYGPPCPPCPAPEFLGGPSVFLFPPKPKDTLMISRTPEVTCVVVDVSQEDPEVQFNWYVDGVEVHNAKTKPREEQFNSTYRVVSVLTVLHQDWLNGKEYKCKVSNKGLPSSIEKTISKAKGQPREPQVYTLPPSQEEMTKNQVSLTCLVKGFYPSDIAVEWESNGQPENNYKTTPPVLDSDGSFFLYSRLTVDKSRWQEGNVFSCSVMHEALHNHYTQKSLSLSLGK

SEQ ID NO: 18 - protein, 445 aa, Artificial Sequence
  humanized
EVQLQESGPGLVKPSETLSLTCTVSGFSLTSNDIAWIRQPPGKGLEWMGTIWTDGSTNYNTAVQSRVTISVDTSKNQFSLKLSSVTAADTAVYYCARHRLYYGAFDYWGQGTMVTVSSASTKGPSVFPLAPCSRSTSESTAALGCLVKDYFPEPVTVSWNSGALTSGVHTFPAVLQSSGLYSLSSVVTVPSSSLGTKTYTCNVDHKPSNTKVDKRVESKYGPPCPPCPAPEFLGGPSVFLFPPKPKDTLMISRTPEVTCVVVDVSQEDPEVQFNWYVDGVEVHNAKTKPREEQFNSTYRVVSVLTVLHQDWLNGKEYKCKVSNKGLPSSIEKTISKAKGQPREPQVYTLPPSQEEMTKNQVSLTCLVKGFYPSDIAVEWESNGQPENNYKTTPPVLDSDGSFFLYSRLTVDKSRWQEGNVFSCSVMHEALHNHYTQKSLSLSLGK

SEQ ID NO: 19 - DNA, 336 bp, Rattus norvegicus
gatattgtgatgacccagactccagtttccctgtctgtcacacttggagatcaagcttctatatcttgcaggtctagtcagagcctggaatatagtgatggctacacttatttggaatggtacctacagaagccaggccagtctcctcagctcctcatctatgaagtttccaaccgattttctggggtcccagacaggttcattggcagtgggtcagggacagatttcaccctcaagatcagcagagtagagcctgaggacttgggagtttattactgcttccaagctacacataatccgtacacgtttggagctgggaccaagctggaaataaaa

SEQ ID NO: 20 - DNA, 354 bp, Rattus norvegicus
gaggtgaagctggaggagtctggacctggcttgatgcagccctcagagaccctgtccctcacctgcactgtctctggcttctcactaaccagcaatgatatagcctgggttcgacaacctctaggaaagggtttggtgtggatgggaacaatatggactgatggaagtacaaattataattcagctgtccaatcccgactgagcatcagcagggacacctccaagagccaatttttcttaaaaatgaacagtctgcaacctgaagacacaggcacttactactgtgccagacatcgcctatactacggggcctttgattactggggccaaggaaccatggtcaccgtctcgagt

SEQ ID NO: 21 - DNA, 336 bp, Artificial Sequence
  humanized
gatatcgtgatgactcagaccccactctcactgtccgtcaccccgggacagcccgcgtcaatctcgtgtaggagctcccaatccctcgaatactcggacggctatacttacctggagtggtacttgcagaagcccggacagagcccgcagcttctgatctacgaagtgtccaacagattctccggcgtgcctgaccgcttttcggggtcgggctccggtactgatttcaccctgaaaatctcccgggtggaagccgaggacgtgggagtctactactgcttccaagccacccacaacccttacaccttcggacaggggaccaagctggagatcaag

SEQ ID NO: 22 - DNA, 354 bp, Artificial Sequence
  humanized
gaggtgcagctgcaggaatccggtcccggcctcgtgaagccttcagaaaccctgtcgctcacatgcactgtgtccgggttctccctgacctctaacgacatcgcctggattcggcagccgccaggaaagggactggagtggatgggcaccatttggaccgacgggtcaaccaactacaatgccgcggtgcaatccagagtgaccatcagcgtggacacgtccaagaaccagttctcgctgaaattgagctccgtgactgccgctgatactgccgtgtattactgtgcccggcaccgcctttactacggcgcatttgactactggggacagggaaccatggtcactgtctcgagt

SEQ ID NO: 23 - DNA, 354 bp, Artificial Sequence
  humanized
gaggtgcaactgcaggaatccggtcccggcctcgtgaagccttcagaaaccctgtcgctcacatgcactgtgtccgggttctccctgacctctaacgacatcgcctggattcggcagccgccaggaaagggactggagtggatgggcaccatttggaccgacgggtcaaccaactacaataccgcggtgcaatccagagtgaccatcagcgtggacacgtccaagaaccagttctcgctgaaattgagctccgtgactgccgctgatactgccgtgtattactgtgcccggcaccgcctttactacggcgcatttgactactggggacagggaaccatggtcactgtctcgagt

SEQ ID NO: 24 - DNA, 657 bp, Artificial Sequence
  humanized
gatatcgtgatgactcagaccccactctcactgtccgtcaccccgggacagcccgcgtcaatctcgtgtaggagctcccaatccctcgaatactcggacggctatacttacctggagtggtacttgcagaagcccggacagagcccgcagcttctgatctacgaagtgtccaacagattctccggcgtgcctgaccgcttttcggggtcgggctccggtactgatttcaccctgaaaatctcccgggtggaagccgaggacgtgggagtctactactgcttccaagccacccacaacccttacaccttcggacaggggaccaagctggagatcaagcggaccgtggccgctccctccgtgttcatcttcccaccctccgacgagcagcttaagtccggcaccgcctccgtcgtgtgcctgctgaacaacttctacccccgcgaggccaaggtgcagtggaaggtggacaacgccctgcagtccggcaactcccaggaatccgtcaccgagcaggactccaaggacagcacctactccctgtcctccaccctgaccctgtccaaggccgactacgagaagcacaaggtgtacgcctgcgaagtgacccaccagggcctgtccagccccgtgaccaagtccttcaaccggggcgagtgc

SEQ ID NO: 25 - DNA, 1335 bp, Artificial Sequence
  humanized
gaggtgcagctgcaggaatccggtcccggcctcgtgaagccttcagaaaccctgtcgctcacatgcactgtgtccgggttctccctgacctctaacgacatcgcctggattcggcagccgccaggaaagggactggagtggatgggcaccatttggaccgacgggtcaaccaactacaatgccgcggtgcaatccagagtgaccatcagcgtggacacgtccaagaaccagttctcgctgaaattgagctccgtgactgccgctgatactgccgtgtattactgtgcccggcaccgcctttactacggcgcatttgactactggggacagggaaccatggtcactgtctcgagtgcctccaccaagggcccctccgtgttccctctggccccttgctcccggtccacctccgagtctaccgccgctctgggctgcctggtcaaggactacttccccgagcccgtgacagtgtcctggaactctggcgccctgacctccggcgtgcacaccttccctgccgtgctgcagtcctccggcctgtactccctgtcctccgtcgtgaccgtgccctcctccagcctgggcaccaagacctacacctgtaacgtggaccacaagccctccaacaccaaggtggacaagcgggtggaatctaagtacggccctccctgccccccctgccctgcccctgaatttctgggcggaccttccgtgttcctgttccccccaaagcccaaggacaccctgatgatctcccggacccccgaagtgacctgcgtggtggtggacgtgtcccaggaagatcccgaggtccagttcaattggtacgtggacggcgtggaagtgcacaatgccaagaccaagcccagagaggaacagttcaactccacctaccgggtggtgtccgtgctgaccgtgctgcaccaggactggctgaacggcaaagagtacaagtgcaaggtgtccaacaagggcctgccctccagcatcgaaaagaccatctccaaggccaagggccagccccgcgagccccaggtgtacaccctgccccctagccaggaagagatgaccaagaaccaggtgtccctgacctgtctggtcaagggcttctacccctccgacattgccgtggaatgggagtccaacggccagcccgagaacaactacaagaccaccccccctgtgctggacagcgacggctccttcttcctgtactctcggctgaccgtggacaagtcccggtggcaggaaggcaacgtcttctcctgctccgtgatgcacgaggccctgcacaaccactacacccagaagtccctgtccctgagcctgggcaag

SEQ ID NO: 26 - DNA, 1335 bp, Artificial Sequence
  humanized
gaggtgcaactgcaggaatccggtcccggcctcgtgaagccttcagaaaccctgtcgctcacatgcactgtgtccgggttctccctgacctctaacgacatcgcctggattcggcagccgccaggaaagggactggagtggatgggcaccatttggaccgacgggtcaaccaactacaataccgcggtgcaatccagagtgaccatcagcgtggacacgtccaagaaccagttctcgctgaaattgagctccgtgactgccgctgatactgccgtgtattactgtgcccggcaccgcctttactacggcgcatttgactactggggacagggaaccatggtcactgtctcgagtgcctccaccaagggcccctccgtgttccctctggccccttgctcccggtccacctccgagtctaccgccgctctgggctgcctggtcaaggactacttccccgagcccgtgacagtgtcctggaactctggcgccctgacctccggcgtgcacaccttccctgccgtgctgcagtcctccggcctgtactccctgtcctccgtcgtgaccgtgccctcctccagcctgggcaccaagacctacacctgtaacgtggaccacaagccctccaacaccaaggtggacaagcgggtggaatctaagtacggccctccctgccccccctgccctgcccctgaatttctgggcggaccttccgtgttcctgttccccccaaagcccaaggacaccctgatgatctcccggacccccgaagtgacctgcgtggtggtggacgtgtcccaggaagatcccgaggtccagttcaattggtacgtggacggcgtggaagtgcacaatgccaagaccaagcccagagaggaacagttcaactccacctaccgggtggtgtccgtgctgaccgtgctgcaccaggactggctgaacggcaaagagtacaagtgcaaggtgtccaacaagggcctgccctccagcatcgaaaagaccatctccaaggccaagggccagccccgcgagccccaggtgtacaccctgccccctagccaggaagagatgaccaagaaccaggtgtccctgacctgtctggtcaagggcttctacccctccgacattgccgtggaatgggagtccaacggccagcccgagaacaactacaagaccaccccccctgtgctggacagcgacggctccttcttcctgtactctcggctgaccgtggacaagtcccggtggcaggaaggcaacgtcttctcctgctccgtgatgcacgaggccctgcacaaccactacacccagaagtccctgtccctgagcctgggcaag

SEQ ID NO: 27 - protein, 134 aa, Rattus norvegicus
  MISC_FEATURE (1)..(22): leader sequence
MDMRVPAQVFGFLLLWFPGTRCDIVMTQTPVSLSVTLGDQASISCRSSQSLEYSDGYTYLEWYLQKPGQSPQLLIYEVSNRFSGVPDRFIGSGSGTDFTLKISRVEPEDLGVYYCFQATHNPYTFGAGTKLEIK

SEQ ID NO: 28 - protein, 136 aa, Rattus norvegicus
MEWSWVFLFFLSVTTGVHSEVKLEESGPGLMQPSETLSLTCTVSGFSLTSNDIAWVRQPLGKGLVWMGTIWTDGSTNYNSAVQSRLSISRDTSKSQFFLKMNSLQPEDTGTYYCARHRLYYGAFDYWGQGTMVTVS

SEQ ID NO: 29 - DNA, 402 bp, Rattus norvegicus
  misc_feature (1)..(66): leader sequence
atggacatgagggttcctgctcaggtttttggcttcttgttgctctggtttccaggcaccaggtgtgatattgtgatgacccagactccagtttccctgtctgtcacacttggagatcaagcttctatatcttgcaggtctagtcagagcctggaatatagtgatggctacacttatttggaatggtacctacagaagccaggccagtctcctcagctcctcatctatgaagtttccaaccgattttctggggtcccagacaggttcattggcagtgggtcagggacagatttcaccctcaagatcagcagagtagagcctgaggacttgggagtttattactgcttccaagctacacataatccgtacacgtttggagctgggaccaagctggaaataaaa

SEQ ID NO: 30 - DNA, 411 bp, Rattus norvegicus
  misc_feature (1)..(57): leader sequence
atggaatggagctgggtctttctcttcttcctgtcagtaactaccggtgtccattctgaggtgaagctggaggagtctggacctggcttgatgcagccctcagagaccctgtccctcacctgcactgtctctggcttctcactaaccagcaatgatatagcctgggttcgacaacctctaggaaagggtttggtgtggatgggaacaatatggactgatggaagtacaaattataattcagctgtccaatcccgactgagcatcagcagggacacctccaagagccaatttttcttaaaaatgaacagtctgcaacctgaagacacaggcacttactactgtgccagacatcgcctatactacggggcctttgattactggggccaaggaaccatggtcaccgtctcgagt

SEQ ID NO: 31 - protein, 112 aa, Homo sapiens
DIVMTQTPLSLSVTPGQPASISCKSSQSLLHSDGKTYLYWYLQKPGQSPQLLIYEVSSRFSGVPDRFSGSGSGTDFTLKISRVEAEDVGVYYCMQGIHLPYTFGQGTKLEIK

SEQ ID NO: 32 - protein, 113 aa, Homo sapiens
QVQLQESGPGLVKPSETLSLTCTVSGGSISSYYWSWIRQPPGKGLEWIGYIYYSGSTNYNPSLKSRVTISVDTSKNQFSLKLSSVTAADTAVYYCARDAFDVWGQGTMVTVSS

SEQ ID NO: 33 - DNA, 336 bp, Homo sapiens
gatattgtgatgacccagactccactctctctgtccgtcacccctggacagccggcctccatctcctgcaagtctagtcagagcctcctgcatagtgatggaaagacctatttgtattggtacctgcagaagccaggccagtctccacagctcctaatctatgaagtttccagccggttctctggagtgccagataggttcagtggcagcgggtcagggacagatttcacactgaaaatcagccgggtggaggctgaggatgttggggtttattactgcatgcaaggtatacaccttccttacacttttggccaggggaccaagctggagatcaaa

SEQ ID NO: 34 - DNA, 339 bp, Homo sapiens
caggtgcagctgcaggagtcgggcccaggactggtgaagccttcggagaccctgtccctcacctgcactgtctctggtggctccatcagtagttactactggagctggatccggcagcccccagggaagggactggagtggattgggtatatctattacagtgggagcaccaactacaacccctccctcaagagtcgagtcaccatatcagtagacacgtccaagaaccagttctccctgaagctgagctctgtgaccgctgcggacacggccgtgtattactgtgcgagagatgcttttgatgtctggggccaagggacaatggtcaccgtctcttca

SEQ ID NO: 35 - protein, 441 aa, Homo sapiens
MAEPRQEFEVMEDHAGTYGLGDRKDQGGYTMHQDQEGDTDAGLKESPLQTPTEDGSEEPGSETSDAKSTPTAEDVTAPLVDEGAPGKQAAAQPHTEIPEGTTAEEAGIGDTPSLEDEAAGHVTQARMVSKSKDGTGSDDKKAKGADGKTKIATPRGAAPPGQKGQANATRIPAKTPPAPKTPPSSGEPPKSGDRSGYSSPGSPGTPGSRSRTPSLPTPPTREPKKVAVVRTPPKSPSSAKSRLQTAPVPMPDLKNVKSKIGSTENLKHQPGGGKVQIINKKLDLSNVQSKCGSKDNIKHVPGGGSVQIVYKPVDLSKVTSKCGSLGNIHHKPGGGQVEVKSEKLDFKDRVQSKIGSLDNITHVPGGGNKKIETHKLTFRENAKAKTDHGAEIVYKSPVVSGDTSPRHLSNVSSTGSIDMVDSPQLATLADEVSASLAKQGL

SEQ ID NO: 36 - protein, 16 aa, Rattus norvegicus
TIWTDGSTNYNSAVQS

SEQ ID NO: 37 - protein, 16 aa, Rattus norvegicus
TIWTDGSTNYNAAVQS

SEQ ID NO: 38 - protein, 16 aa, Rattus norvegicus
TIWTDGSTNYNTAVQS

SEQ ID NO: 39 - DNA, 6757 bp, Artificial Sequence
  synthetic
tggcgaatgggacgcgccctgtagcggcgcattaagcgcggcgggtgtggtggttacgcgcagcgtgaccgctacacttgccagcgccctagcgcccgctcctttcgctttcttcccttcctttctcgccacgttcgccggctttccccgtcaagctctaaatcgggggctccctttagggttccgatttagtgctttacggcacctcgaccccaaaaaacttgattagggtgatggttcacgtagtgggccatcgccctgatagacggtttttcgccctttgacgttggagtccacgttctttaatagtggactcttgttccaaactggaacaacactcaaccctatctcggtctattcttttgatttataagggattttgccgatttcggcctattggttaaaaaatgagctgatttaacaaaaatttaacgcgaattttaacaaaatattaacgtttacaatttcaggtggcacttttcggggaaatgtgcgcggaacccctatttgtttatttttctaaatacattcaaatatgtatccgctcatgagacaataaccctgataaatgcttcaataatattgaaaaaggaagagtatgagtattcaacatttccgtgtcgcccttattcccttttttgcggcattttgccttcctgtttttgctcacccagaaacgctggtgaaagtaaaagatgctgaagatcagttgggtgcacgagtgggttacatcgaactggatctcaacagcggtaagatccttgagagttttcgccccgaagaacgttttccaatgatgagcacttttaaagttctgctatgtggcgcggtattatcccgtattgacgccgggcaagagcaactcggtcgccgcatacactattctcagaatgacttggttgagtactcaccagtcacagaaaagcatcttacggatggcatgacagtaagagaattatgcagtgctgccataaccatgagtgataacactgcggccaacttacttctgacaacgatcggaggaccgaaggagctaaccgcttttttgcacaacatgggggatcatgtaactcgccttgatcgttgggaaccggagctgaatgaagccataccaaacgacgagcgtgacaccacgatgcctgcagcaatggcaacaacgttgcgcaaactattaactggcgaactacttactctagcttcccggcaacaattaatagactggatggaggcggataaagttgcaggaccacttctgcgctcggcccttccggctggctggtttattgctgataaatctggagccggtgagcgtgggtctcgcggtatcattgcagcactggggccagatggtaagccctcccgtatcgtagttatctacacgacggggagtcaggcaactatggatgaacgaaatagacagatcgctgagataggtgcctcactgattaagcattggtaactgtcagaccaagtttactcatatatactttagattgatttaaaacttcatttttaatttaaaaggatctaggtgaagatcctttttgataatctcatgaccaaaatcccttaacgtgagttttcgttccactgagcgtcagaccccgtagaaaagatcaaaggatcttcttgagatcctttttttctgcgcgtaatctgctgcttgcaaacaaaaaaaccaccgctaccagcggtggtttgtttgccggatcaagagctaccaactctttttccgaaggtaactggcttcagcagagcgcagataccaaatactgtccttctagtgtagccgtagttaggccaccacttcaagaactctgtagcaccgcctacatacctcgctctgctaatcctgttaccagtggctgctgccagtggcgataagtcgtgtcttaccgggttggactcaagacgatagttaccggataaggcgcagcggtcgggctgaacggggggttcgtgcacacagcccagcttggagcgaacgacctacaccgaactgagatacctacagcgtgagctatgagaaagcgccacgcttcccgaagggagaaaggcggacaggtatccggtaagcggcagggtcggaacaggagagcgcacgagggagcttccagggggaaacgcctggtatctttatagtcctgtcgggtttcgccacctctgacttgagcgtcgatttttgtgatgctcgtcaggggggcggagcctatggaaaaacgccagcaacgcggcctttttacggttcctggccttttgctggccttttgctcacatgttctttcctgcgttatcccctgattctgtggataaccgtattaccgcctttgagtgagctgataccgctcgccgcagccgaacgaccgagcgcagcgagtcagtgagcgaggaagcggaagagcgcctgatgcggtattttctccttacgcatctgtgcggtatttcacaccgcatatatggtgcactctcagtacaatctgctctgatgccgcatagttaagccagtatacactccgctatcgctacgtgactgggtcatggctgcgccccgacacccgccaacacccgctgacgcgccctgacgggcttgtctgctcccggcatccgcttacagacaagctgtgaccgtctccgggagctgcatgtgtcagaggttttcaccgtcatcaccgaaacgcgcgaggcagctgcggtaaagctcatcagcgtggtcgtgaagcgattcacagatgtctgcctgttcatccgcgtccagctcgttgagtttctccagaagcgttaatgtctggcttctgataaagcgggccatgttaagggcggttttttcctgtttggtcactgatgcctccgtgtaagggggatttctgttcatgggggtaatgataccgatgaaacgagagaggatgctcacgatacgggttactgatgatgaacatgcccggttactggaacgttgtgagggtaaacaactggcggtatggatgcggcgggaccagagaaaaatcactcagggtcaatgccagcgcttcgttaatacagatgtaggtgttccacagggtagccagcagcatcctgcgatgcagatccggaacataatggtgcagggcgctgacttccgcgtttccagactttacgaaacacggaaaccgaagaccattcatgttgttgctcaggtcgcagacgttttgcagcagcagtcgcttcacgttcgctcgcgtatcggtgattcattctgctaaccagtaaggcaaccccgccagcctagccgggtcctcaacgacaggagcacgatcatgcgcacccgtggggccgccatgccggcgataatggcctgcttctcgccgaaacgtttggtggcgggaccagtgacgaaggcttgagcgagggcgtgcaagattccgaataccgcaagcgacaggccgatcatcgtcgcgctccagcgaaagcggtcctcgccgaaaatgacccagagcgctgccggcacctgtcctacgagttgcatgataaagaagacagtcataagtgcggcgacgatagtcatgccccgcgcccaccggaaggagctgactgggttgaaggctctcaagggcatcggtcgagatcccggtgcctaatgagtgagctaacttacattaattgcgttgcgctcactgcccgctttccagtcgggaaacctgtcgtgccagctgcattaatgaatcggccaacgcgcggggagaggcggtttgcgtattgggcgccagggtggtttttcttttcaccagtgagacgggcaacagctgattgcccttcaccgcctggccctgagagagttgcagcaagcggtccacgctggtttgccccagcaggcgaaaatcctgtttgatggtggttaacggcgggatataacatgagctgtcttcggtatcgtcgtatcccactaccgagatgtccgcaccaacgcgcagcccggactcggtaatggcgcgcattgcgcccagcgccatctgatcgttggcaaccagcatcgcagtgggaacgatgccctcattcagcatttgcatggtttgttgaaaaccggacatggcactccagtcgccttcccgttccgctatcggctgaatttgattgcgagtgagatatttatgccagccagccagacgcagacgcgccgagacagaacttaatgggcccgctaacagcgcgatttgctggtgacccaatgcgaccagatgctccacgcccagtcgcgtaccgtcttcatgggagaaaataatactgttgatgggtgtctggtcagagacatcaagaaataacgccggaacattagtgcaggcagcttccacagcaatggcatcctggtcatccagcggatagttaatgatcagcccactgacgcgttgcgcgagaagattgtgcaccgccgctttacaggcttcgacgccgcttcgttctaccatcgacaccaccacgctggcacccagttgatcggcgcgagatttaatcgccgcgacaatttgcgacggcgcgtgcagggccagactggaggtggcaacgccaatcagcaacgactgtttgcccgccagttgttgtgccacgcggttgggaatgtaattcagctccgccatcgccgcttccactttttcccgcgttttcgcagaaacgtggctggcctggttcaccacgcgggaaacggtctgataagagacaccggcatactctgcgacatcgtataacgttactggtttcacattcaccaccctgaattgactctcttccgggcgctatcatgccataccgcgaaaggttttgcgccattcgatggtgtccgggatctcgacgctctcccttatgcgactcctgcattaggaagcagcccagtagtaggttgaggccgttgagcaccgccgccgcaaggaatggtgcatgcaaggagatggcgcccaacagtcccccggccacggggcctgccaccatacccacgccgaaacaagcgctcatgagcccgaagtggcgagcccgatcttccccatcggtgatgtcggcgatataggcgccagcaaccgcacctgtggcgccggtgatgccggccacgatgcgtccggcgtagaggatcgagatcgatctcgatcccgcgaaattaatacgactcactataggggaattgtgagcggataacaattcccctctagaaataattttgtttaactttaagaaggagatatacatatgggctcaagccaccaccaccaccaccacagcagcggcgagaacttgtactttcaaggatccgcagaaccacgtcaagaatttgaggttatggaagatcacgcgggcacttacggtttgggtgatcgtaaagaccagggcggctataccatgcatcaagatcaagagggcgacaccgatgctggcttgaaagagtcgccgctgcagactccgaccgaggatggcagcgaagagccgggcagcgagactagcgatgcgaagtcgaccccgaccgccgaggacgttaccgcaccgctggtcgacgagggtgctccgggtaaacaggcggctgcacagccgcacacggagattccggaaggcaccaccgcagaagaggcgggtatcggcgacactccgtccctggaagatgaggcagccggtcatgtcacgcaggcgcgtatggtgagcaagagcaaagatggtacgggtagcgacgacaagaaggcgaagggcgcagatggcaagaccaaaattgcgacgccgcgtggtgcggcaccgccaggccagaaaggtcaggcgaatgccacgcgcatcccggcaaagacgccaccggctccgaaaaccccgccttccagcggtgaaccgccgaaatccggtgaccgcagcggttatagctctccgggtagcccgggtaccccaggcagccgtagccgcaccccgagcctgccgaccccaccgacccgcgagccgaagaaagtggcggtggttcgtacgccgccaaaaagcccgagctctgccaagagccgtctgcaaaccgctcctgtgccgatgccggacctgaagaacgttaagtctaaaatcggtagcaccgaaaatctgaagcaccaacctggtggcggtaaggttcaaatcatcaacaaaaagctggacttgagcaatgtacaaagcaagtgtggtagcaaggacaatatcaaacacgtcccgggtggtggttccgtccagattgtgtacaaaccggtggacctgagcaaggttaccagcaaatgcggttccctgggtaacatccatcataaaccgggtggcggccaagttgaggtcaagagcgagaaactggacttcaaagaccgcgttcagtccaaaatcggttctctggacaacattacgcacgtgcctggtggtggcaacaagaagattgaaacccataaactgacgtttcgtgaaaatgcgaaggcgaaaaccgaccacggcgcagagattgtctacaaaagcccggtggtgagcggtgataccagcccgcgtcacctgtccaacgtcagcagcacgggcagcattgatatggtggatagcccgcagttggctacgctggccgatgaggttagcgcgagcctggcgaagcagggtctgtgactcgagcaccaccaccaccaccactgagatccggctgctaacaaagcccgaaaggaagctgagttggctgctgccaccgctgagcaataactagcataaccccttggggcctctaaacgggtcttgaggggttttttgctgaaaggaggaactatatccggat

SEQ ID NO: 40 - protein, 461 aa, Artificial Sequence
  synthetic
MGSSHHHHHHSSGENLYFQGSAEPRQEFEVMEDHAGTYGLGDRKDQGGYTMHQDQEGDTDAGLKESPLQTPTEDGSEEPGSETSDAKSTPTAEDVTAPLVDEGAPGKQAAAQPHTEIPEGTTAEEAGIGDTPSLEDEAAGHVTQARMVSKSKDGTGSDDKKAKGADGKTKIATPRGAAPPGQKGQANATRIPAKTPPAPKTPPSSGEPPKSGDRSGYSSPGSPGTPGSRSRTPSLPTPPTREPKKVAVVRTPPKSPSSAKSRLQTAPVPMPDLKNVKSKIGSTENLKHQPGGGKVQIINKKLDLSNVQSKCGSKDNIKHVPGGGSVQIVYKPVDLSKVTSKCGSLGNIHHKPGGGQVEVKSEKLDFKDRVQSKIGSLDNITHVPGGGNKKIETHKLTFRENAKAKTDHGAEIVYKSPVVSGDTSPRHLSNVSSTGSIDMVDSPQLATLADEVSASLAKQGL

SEQ ID NO: 41 - protein, 442 aa, Artificial Sequence
  synthetic
GSAEPRQEFEVMEDHAGTYGLGDRKDQGGYTMHQDQEGDTDAGLKESPLQTPTEDGSEEPGSETSDAKSTPTAEDVTAPLVDEGAPGKQAAAQPHTEIPEGTTAEEAGIGDTPSLEDEAAGHVTQARMVSKSKDGTGSDDKKAKGADGKTKIATPRGAAPPGQKGQANATRIPAKTPPAPKTPPSSGEPPKSGDRSGYSSPGSPGTPGSRSRTPSLPTPPTREPKKVAVVRTPPKSPSSAKSRLQTAPVPMPDLKNVKSKIGSTENLKHQPGGGKVQIINKKLDLSNVQSKCGSKDNIKHVPGGGSVQIVYKPVDLSKVTSKCGSLGNIHHKPGGGQVEVKSEKLDFKDRVQSKIGSLDNITHVPGGGNKKIETHKLTFRENAKAKTDHGAEIVYKSPVVSGDTSPRHLSNVSSTGSIDMVDSPQLATLADEVSASLAKQGL

SEQ ID NO: 42 - DNA, 6583 bp, Artificial Sequence
  synthetic
tggcgaatgggacgcgccctgtagcggcgcattaagcgcggcgggtgtggtggttacgcgcagcgtgaccgctacacttgccagcgccctagcgcccgctcctttcgctttcttcccttcctttctcgccacgttcgccggctttccccgtcaagctctaaatcgggggctccctttagggttccgatttagtgctttacggcacctcgaccccaaaaaacttgattagggtgatggttcacgtagtgggccatcgccctgatagacggtttttcgccctttgacgttggagtccacgttctttaatagtggactcttgttccaaactggaacaacactcaaccctatctcggtctattcttttgatttataagggattttgccgatttcggcctattggttaaaaaatgagctgatttaacaaaaatttaacgcgaattttaacaaaatattaacgtttacaatttcaggtggcacttttcggggaaatgtgcgcggaacccctatttgtttatttttctaaatacattcaaatatgtatccgctcatgagacaataaccctgataaatgcttcaataatattgaaaaaggaagagtatgagtattcaacatttccgtgtcgcccttattcccttttttgcggcattttgccttcctgtttttgctcacccagaaacgctggtgaaagtaaaagatgctgaagatcagttgggtgcacgagtgggttacatcgaactggatctcaacagcggtaagatccttgagagttttcgccccgaagaacgttttccaatgatgagcacttttaaagttctgctatgtggcgcggtattatcccgtattgacgccgggcaagagcaactcggtcgccgcatacactattctcagaatgacttggttgagtactcaccagtcacagaaaagcatcttacggatggcatgacagtaagagaattatgcagtgctgccataaccatgagtgataacactgcggccaacttacttctgacaacgatcggaggaccgaaggagctaaccgcttttttgcacaacatgggggatcatgtaactcgccttgatcgttgggaaccggagctgaatgaagccataccaaacgacgagcgtgacaccacgatgcctgcagcaatggcaacaacgttgcgcaaactattaactggcgaactacttactctagcttcccggcaacaattaatagactggatggaggcggataaagttgcaggaccacttctgcgctcggcccttccggctggctggtttattgctgataaatctggagccggtgagcgtgggtctcgcggtatcattgcagcactggggccagatggtaagccctcccgtatcgtagttatctacacgacggggagtcaggcaactatggatgaacgaaatagacagatcgctgagataggtgcctcactgattaagcattggtaactgtcagaccaagtttactcatatatactttagattgatttaaaacttcatttttaatttaaaaggatctaggtgaagatcctttttgataatctcatgaccaaaatcccttaacgtgagttttcgttccactgagcgtcagaccccgtagaaaagatcaaaggatcttcttgagatcctttttttctgcgcgtaatctgctgcttgcaaacaaaaaaaccaccgctaccagcggtggtttgtttgccggatcaagagctaccaactctttttccgaaggtaactggcttcagcagagcgcagataccaaatactgtccttctagtgtagccgtagttaggccaccacttcaagaactctgtagcaccgcctacatacctcgctctgctaatcctgttaccagtggctgctgccagtggcgataagtcgtgtcttaccgggttggactcaagacgatagttaccggataaggcgcagcggtcgggctgaacggggggttcgtgcacacagcccagcttggagcgaacgacctacaccgaactgagatacctacagcgtgagctatgagaaagcgccacgcttcccgaagggagaaaggcggacaggtatccggtaagcggcagggtcggaacaggagagcgcacgagggagcttccagggggaaacgcctggtatctttatagtcctgtcgggtttcgccacctctgacttgagcgtcgatttttgtgatgctcgtcaggggggcggagcctatggaaaaacgccagcaacgcggcctttttacggttcctggccttttgctggccttttgctcacatgttctttcctgcgttatcccctgattctgtggataaccgtattaccgcctttgagtgagctgataccgctcgccgcagccgaacgaccgagcgcagcgagtcagtgagcgaggaagcggaagagcgcctgatgcggtattttctccttacgcatctgtgcggtatttcacaccgcatatatggtgcactctcagtacaatctgctctgatgccgcatagttaagccagtatacactccgctatcgctacgtgactgggtcatggctgcgccccgacacccgccaacacccgctgacgcgccctgacgggcttgtctgctcccggcatccgcttacagacaagctgtgaccgtctccgggagctgcatgtgtcagaggttttcaccgtcatcaccgaaacgcgcgaggcagctgcggtaaagctcatcagcgtggtcgtgaagcgattcacagatgtctgcctgttcatccgcgtccagctcgttgagtttctccagaagcgttaatgtctggcttctgataaagcgggccatgttaagggcggttttttcctgtttggtcactgatgcctccgtgtaagggggatttctgttcatgggggtaatgataccgatgaaacgagagaggatgctcacgatacgggttactgatgatgaacatgcccggttactggaacgttgtgagggtaaacaactggcggtatggatgcggcgggaccagagaaaaatcactcagggtcaatgccagcgcttcgttaatacagatgtaggtgttccacagggtagccagcagcatcctgcgatgcagatccggaacataatggtgcagggcgctgacttccgcgtttccagactttacgaaacacggaaaccgaagaccattcatgttgttgctcaggtcgcagacgttttgcagcagcagtcgcttcacgttcgctcgcgtatcggtgattcattctgctaaccagtaaggcaaccccgccagcctagccgggtcctcaacgacaggagcacgatcatgcgcacccgtggggccgccatgccggcgataatggcctgcttctcgccgaaacgtttggtggcgggaccagtgacgaaggcttgagcgagggcgtgcaagattccgaataccgcaagcgacaggccgatcatcgtcgcgctccagcgaaagcggtcctcgccgaaaatgacccagagcgctgccggcacctgtcctacgagttgcatgataaagaagacagtcataagtgcggcgacgatagtcatgccccgcgcccaccggaaggagctgactgggttgaaggctctcaagggcatcggtcgagatcccggtgcctaatgagtgagctaacttacattaattgcgttgcgctcactgcccgctttccagtcgggaaacctgtcgtgccagctgcattaatgaatcggccaacgcgcggggagaggcggtttgcgtattgggcgccagggtggtttttcttttcaccagtgagacgggcaacagctgattgcccttcaccgcctggccctgagagagttgcagcaagcggtccacgctggtttgccccagcaggcgaaaatcctgtttgatggtggttaacggcgggatataacatgagctgtcttcggtatcgtcgtatcccactaccgagatgtccgcaccaacgcgcagcccggactcggtaatggcgcgcattgcgcccagcgccatctgatcgttggcaaccagcatcgcagtgggaacgatgccctcattcagcatttgcatggtttgttgaaaaccggacatggcactccagtcgccttcccgttccgctatcggctgaatttgattgcgagtgagatatttatgccagccagccagacgcagacgcgccgagacagaacttaatgggcccgctaacagcgcgatttgctggtgacccaatgcgaccagatgctccacgcccagtcgcgtaccgtcttcatgggagaaaataatactgttgatgggtgtctggtcagagacatcaagaaataacgccggaacattagtgcaggcagcttccacagcaatggcatcctggtcatccagcggatagttaatgatcagcccactgacgcgttgcgcgagaagattgtgcaccgccgctttacaggcttcgacgccgcttcgttctaccatcgacaccaccacgctggcacccagttgatcggcgcgagatttaatcgccgcgacaatttgcgacggcgcgtgcagggccagactggaggtggcaacgccaatcagcaacgactgtttgcccgccagttgttgtgccacgcggttgggaatgtaattcagctccgccatcgccgcttccactttttcccgcgttttcgcagaaacgtggctggcctggttcaccacgcgggaaacggtctgataagagacaccggcatactctgcgacatcgtataacgttactggtttcacattcaccaccctgaattgactctcttccgggcgctatcatgccataccgcgaaaggttttgcgccattcgatggtgtccgggatctcgacgctctcccttatgcgactcctgcattaggaagcagcccagtagtaggttgaggccgttgagcaccgccgccgcaaggaatggtgcatgcaaggagatggcgcccaacagtcccccggccacggggcctgccaccatacccacgccgaaacaagcgctcatgagcccgaagtggcgagcccgatcttccccatcggtgatgtcggcgatataggcgccagcaaccgcacctgtggcgccggtgatgccggccacgatgcgtccggcgtagaggatcgagatcgatctcgatcccgcgaaattaatacgactcactataggggaattgtgagcggataacaattcccctctagaaataattttgtttaactttaagaaggagatatacatatgggctcaagccaccaccaccaccaccacagcagcggcgagaacttgtactttcaaggatccgcagaaccacgtcaagaatttgaggttatggaagatcacgcgggcacttacggtttgggtgatcgtaaagaccagggcggctataccatgcatcaagatcaagagggcgacaccgatgctggcttgaaagcagaagaggcgggtatcggcgacactccgtccctggaagatgaggcagccggtcatgtcacgcaggcgcgtatggtgagcaagagcaaagatggtacgggtagcgacgacaagaaggcgaagggcgcagatggcaagaccaaaattgcgacgccgcgtggtgcggcaccgccaggccagaaaggtcaggcgaatgccacgcgcatcccggcaaagacgccaccggctccgaaaaccccgccttccagcggtgaaccgccgaaatccggtgaccgcagcggttatagctctccgggtagcccgggtaccccaggcagccgtagccgcaccccgagcctgccgaccccaccgacccgcgagccgaagaaagtggcggtggttcgtacgccgccaaaaagcccgagctctgccaagagccgtctgcaaaccgctcctgtgccgatgccggacctgaagaacgttaagtctaaaatcggtagcaccgaaaatctgaagcaccaacctggtggcggtaaggttcaaatcatcaacaaaaagctggacttgagcaatgtacaaagcaagtgtggtagcaaggacaatatcaaacacgtcccgggtggtggttccgtccagattgtgtacaaaccggtggacctgagcaaggttaccagcaaatgcggttccctgggtaacatccatcataaaccgggtggcggccaagttgaggtcaagagcgagaaactggacttcaaagaccgcgttcagtccaaaatcggttctctggacaacattacgcacgtgcctggtggtggcaacaagaagattgaaacccataaactgacgtttcgtgaaaatgcgaaggcgaaaaccgaccacggcgcagagattgtctacaaaagcccggtggtgagcggtgataccagcccgcgtcacctgtccaacgtcagcagcacgggcagcattgatatggtggatagcccgcagttggctacgctggccgatgaggttagcgcgagcctggcgaagcagggtctgtgactcgagcaccaccaccaccaccactgagatccggctgctaacaaagcccgaaaggaagctgagttggctgctgccaccgctgagcaataactagcataaccccttggggcctctaaacgggtcttgaggggttttttgctgaaaggaggaactatatccggat

SEQ ID NO: 43 - protein, 403 aa, Artificial Sequence
  synthetic
MGSSHHHHHHSSGENLYFQGSAEPRQEFEVMEDHAGTYGLGDRKDQGGYTMHQDQEGDTDAGLKAEEAGIGDTPSLEDEAAGHVTQARMVSKSKDGTGSDDKKAKGADGKTKIATPRGAAPPGQKGQANATRIPAKTPPAPKTPPSSGEPPKSGDRSGYSSPGSPGTPGSRSRTPSLPTPPTREPKKVAVVRTPPKSPSSAKSRLQTAPVPMPDLKNVKSKIGSTENLKHQPGGGKVQIINKKLDLSNVQSKCGSKDNIKHVPGGGSVQIVYKPVDLSKVTSKCGSLGNIHHKPGGGQVEVKSEKLDFKDRVQSKIGSLDNITHVPGGGNKKIETHKLTFRENAKAKTDHGAEIVYKSPVVSGDTSPRHLSNVSSTGSIDMVDSPQLATLADEVSASLAKQGL

SEQ ID NO: 44 - protein, 384 aa, Artificial Sequence
  synthetic
GSAEPRQEFEVMEDHAGTYGLGDRKDQGGYTMHQDQEGDTDAGLKAEEAGIGDTPSLEDEAAGHVTQARMVSKSKDGTGSDDKKAKGADGKTKIATPRGAAPPGQKGQANATRIPAKTPPAPKTPPSSGEPPKSGDRSGYSSPGSPGTPGSRSRTPSLPTPPTREPKKVAVVRTPPKSPSSAKSRLQTAPVPMPDLKNVKSKIGSTENLKHQPGGGKVQIINKKLDLSNVQSKCGSKDNIKHVPGGGSVQIVYKPVDLSKVTSKCGSLGNIHHKPGGGQVEVKSEKLDFKDRVQSKIGSLDNITHVPGGGNKKIETHKLTFRENAKAKTDHGAEIVYKSPVVSGDTSPRHLSNVSSTGSIDMVDSPQLATLADEVSASLAKQGL

SEQ ID NO: 45 - DNA, 6490 bp, Artificial Sequence
  synthetic
tggcgaatgggacgcgccctgtagcggcgcattaagcgcggcgggtgtggtggttacgcgcagcgtgaccgctacacttgccagcgccctagcgcccgctcctttcgctttcttcccttcctttctcgccacgttcgccggctttccccgtcaagctctaaatcgggggctccctttagggttccgatttagtgctttacggcacctcgaccccaaaaaacttgattagggtgatggttcacgtagtgggccatcgccctgatagacggtttttcgccctttgacgttggagtccacgttctttaatagtggactcttgttccaaactggaacaacactcaaccctatctcggtctattcttttgatttataagggattttgccgatttcggcctattggttaaaaaatgagctgatttaacaaaaatttaacgcgaattttaacaaaatattaacgtttacaatttcaggtggcacttttcggggaaatgtgcgcggaacccctatttgtttatttttctaaatacattcaaatatgtatccgctcatgagacaataaccctgataaatgcttcaataatattgaaaaaggaagagtatgagtattcaacatttccgtgtcgcccttattcccttttttgcggcattttgccttcctgtttttgctcacccagaaacgctggtgaaagtaaaagatgctgaagatcagttgggtgcacgagtgggttacatcgaactggatctcaacagcggtaagatccttgagagttttcgccccgaagaacgttttccaatgatgagcacttttaaagttctgctatgtggcgcggtattatcccgtattgacgccgggcaagagcaactcggtcgccgcatacactattctcagaatgacttggttgagtactcaccagtcacagaaaagcatcttacggatggcatgacagtaagagaattatgcagtgctgccataaccatgagtgataacactgcggccaacttacttctgacaacgatcggaggaccgaaggagctaaccgcttttttgcacaacatgggggatcatgtaactcgccttgatcgttgggaaccggagctgaatgaagccataccaaacgacgagcgtgacaccacgatgcctgcagcaatggcaacaacgttgcgcaaactattaactggcgaactacttactctagcttcccggcaacaattaatagactggatggaggcggataaagttgcaggaccacttctgcgctcggcccttccggctggctggtttattgctgataaatctggagccggtgagcgtgggtctcgcggtatcattgcagcactggggccagatggtaagccctcccgtatcgtagttatctacacgacggggagtcaggcaactatggatgaacgaaatagacagatcgctgagataggtgcctcactgattaagcattggtaactgtcagaccaagtttactcatatatactttagattgatttaaaacttcatttttaatttaaaaggatctaggtgaagatcctttttgataatctcatgaccaaaatcccttaacgtgagttttcgttccactgagcgtcagaccccgtagaaaagatcaaaggatcttcttgagatcctttttttctgcgcgtaatctgctgcttgcaaacaaaaaaaccaccgctaccagcggtggtttgtttgccggatcaagagctaccaactctttttccgaaggtaactggcttcagcagagcgcagataccaaatactgtccttctagtgtagccgtagttaggccaccacttcaagaactctgtagcaccgcctacatacctcgctctgctaatcctgttaccagtggctgctgccagtggcgataagtcgtgtcttaccgggttggactcaagacgatagttaccggataaggcgcagcggtcgggctgaacggggggttcgtgcacacagcccagcttggagcgaacgacctacaccgaactgagatacctacagcgtgagctatgagaaagcgccacgcttcccgaagggagaaaggcggacaggtatccggtaagcggcagggtcggaacaggagagcgcacgagggagcttccagggggaaacgcctggtatctttatagtcctgtcgggtttcgccacctctgacttgagcgtcgatttttgtgatgctcgtcaggggggcggagcctatggaaaaacgccagcaacgcggcctttttacggttcctggccttttgctggccttttgctcacatgttctttcctgcgttatcccctgattctgtggataaccgtattaccgcctttgagtgagctgataccgctcgccgcagccgaacgaccgagcgcagcgagtcagtgagcgaggaagcggaagagcgcctgatgcggtattttctccttacgcatctgtgcggtatttcacaccgcatatatggtgcactctcagtacaatctgctctgatgccgcatagttaagccagtatacactccgctatcgctacgtgactgggtcatggctgcgccccgacacccgccaacacccgctgacgcgccctgacgggcttgtctgctcccggcatccgcttacagacaagctgtgaccgtctccgggagctgcatgtgtcagaggttttcaccgtcatcaccgaaacgcgcgaggcagctgcggtaaagctcatcagcgtggtcgtgaagcgattcacagatgtctgcctgttcatccgcgtccagctcgttgagtttctccagaagcgttaatgtctggcttctgataaagcgggccatgttaagggcggttttttcctgtttggtcactgatgcctccgtgtaagggggatttctgttcatgggggtaatgataccgatgaaacgagagaggatgctcacgatacgggttactgatgatgaacatgcccggttactggaacgttgtgagggtaaacaactggcggtatggatgcggcgggaccagagaaaaatcactcagggtcaatgccagcgcttcgttaatacagatgtaggtgttccacagggtagccagcagcatcctgcgatgcagatccggaacataatggtgcagggcgctgacttccgcgtttccagactttacgaaacacggaaaccgaagaccattcatgttgttgctcaggtcgcagacgttttgcagcagcagtcgcttcacgttcgctcgcgtatcggtgattcattctgctaaccagtaaggcaaccccgccagcctagccgggtcctcaacgacaggagcacgatcatgcgcacccgtggggccgccatgccggcgataatggcctgcttctcgccgaaacgtttggtggcgggaccagtgacgaaggcttgagcgagggcgtgcaagattccgaataccgcaagcgacaggccgatcatcgtcgcgctccagcgaaagcggtcctcgccgaaaatgacccagagcgctgccggcacctgtcctacgagttgcatgataaagaagacagtcataagtgcggcgacgatagtcatgccccgcgcccaccggaaggagctgactgggttgaaggctctcaagggcatcggtcgagatcccggtgcctaatgagtgagctaacttacattaattgcgttgcgctcactgcccgctttccagtcgggaaacctgtcgtgccagctgcattaatgaatcggccaacgcgcggggagaggcggtttgcgtattgggcgccagggtggtttttcttttcaccagtgagacgggcaacagctgattgcccttcaccgcctggccctgagagagttgcagcaagcggtccacgctggtttgccccagcaggcgaaaatcctgtttgatggtggttaacggcgggatataacatgagctgtcttcggtatcgtcgtatcccactaccgagatgtccgcaccaacgcgcagcccggactcggtaatggcgcgcattgcgcccagcgccatctgatcgttggcaaccagcatcgcagtgggaacgatgccctcattcagcatttgcatggtttgttgaaaaccggacatggcactccagtcgccttcccgttccgctatcggctgaatttgattgcgagtgagatatttatgccagccagccagacgcagacgcgccgagacagaacttaatgggcccgctaacagcgcgatttgctggtgacccaatgcgaccagatgctccacgcccagtcgcgtaccgtcttcatgggagaaaataatactgttgatgggtgtctggtcagagacatcaagaaataacgccggaacattagtgcaggcagcttccacagcaatggcatcctggtcatccagcggatagttaatgatcagcccactgacgcgttgcgcgagaagattgtgcaccgccgctttacaggcttcgacgccgcttcgttctaccatcgacaccaccacgctggcacccagttgatcggcgcgagatttaatcgccgcgacaatttgcgacggcgcgtgcagggccagactggaggtggcaacgccaatcagcaacgactgtttgcccgccagttgttgtgccacgcggttgggaatgtaattcagctccgccatcgccgcttccactttttcccgcgttttcgcagaaacgtggctggcctggttcaccacgcgggaaacggtctgataagagacaccggcatactctgcgacatcgtataacgttactggtttcacattcaccaccctgaattgactctcttccgggcgctatcatgccataccgcgaaaggttttgcgccattcgatggtgtccgggatctcgacgctctcccttatgcgactcctgcattaggaagcagcccagtagtaggttgaggccgttgagcaccgccgccgcaaggaatggtgcatgcaaggagatggcgcccaacagtcccccggccacggggcctgccaccatacccacgccgaaacaagcgctcatgagcccgaagtggcgagcccgatcttccccatcggtgatgtcggcgatataggcgccagcaaccgcacctgtggcgccggtgatgccggccacgatgcgtccggcgtagaggatcgagatcgatctcgatcccgcgaaattaatacgactcactataggggaattgtgagcggataacaattcccctctagaaataattttgtttaactttaagaaggagatatacatatgggctcaagccaccaccaccaccaccacagcagcggcgagaacttgtactttcaaggatccgcagaaccacgtcaagaatttgaggttatggaagatcacgcgggcacttacggtttgggtgatcgtaaagaccagggcggctataccatgcatcaagatcaagagggcgacaccgatgctggcttgaaagcagaagaggcgggtatcggcgacactccgtccctggaagatgaggcagccggtcatgtcacgcaggcgcgtatggtgagcaagagcaaagatggtacgggtagcgacgacaagaaggcgaagggcgcagatggcaagaccaaaattgcgacgccgcgtggtgcggcaccgccaggccagaaaggtcaggcgaatgccacgcgcatcccggcaaagacgccaccggctccgaaaaccccgccttccagcggtgaaccgccgaaatccggtgaccgcagcggttatagctctccgggtagcccgggtaccccaggcagccgtagccgcaccccgagcctgccgaccccaccgacccgcgagccgaagaaagtggcggtggttcgtacgccgccaaaaagcccgagctctgccaagagccgtctgcaaaccgctcctgtgccgatgccggacctgaagaacgttaagtctaaaatcggtagcaccgaaaatctgaagcaccaacctggtggcggtaaggtccagattgtgtacaaaccggtggacctgagcaaggttaccagcaaatgcggttccctgggtaacatccatcataaaccgggtggcggccaagttgaggtcaagagcgagaaactggacttcaaagaccgcgttcagtccaaaatcggttctctggacaacattacgcacgtgcctggtggtggcaacaagaagattgaaacccataaactgacgtttcgtgaaaatgcgaaggcgaaaaccgaccacggcgcagagattgtctacaaaagcccggtggtgagcggtgataccagcccgcgtcacctgtccaacgtcagcagcacgggcagcattgatatggtggatagcccgcagttggctacgctggccgatgaggttagcgcgagcctggcgaagcagggtctgtgactcgagcaccaccaccaccaccactgagatccggctgctaacaaagcccgaaaggaagctgagttggctgctgccaccgctgagcaataactagcataaccccttggggcctctaaacgggtcttgaggggttttttgctgaaaggaggaactatatccggat

SEQ ID NO: 46 - protein, 372 aa, Artificial Sequence
  synthetic
MGSSHHHHHHSSGENLYFQGSAEPRQEFEVMEDHAGTYGLGDRKDQGGYTMHQDQEGDTDAGLKAEEAGIGDTPSLEDEAAGHVTQARMVSKSKDGTGSDDKKAKGADGKTKIATPRGAAPPGQKGQANATRIPAKTPPAPKTPPSSGEPPKSGDRSGYSSPGSPGTPGSRSRTPSLPTPPTREPKKVAVVRTPPKSPSSAKSRLQTAPVPMPDLKNVKSKIGSTENLKHQPGGGKVQIVYKPVDLSKVTSKCGSLGNIHHKPGGGQVEVKSEKLDFKDRVQSKIGSLDNITHVPGGGNKKIETHKLTFRENAKAKTDHGAEIVYKSPVVSGDTSPRHLSNVSSTGSIDMVDSPQLATLADEVSASLAKQGL

SEQ ID NO: 47 - protein, 353 aa, Artificial Sequence
  synthetic
GSAEPRQEFEVMEDHAGTYGLGDRKDQGGYTMHQDQEGDTDAGLKAEEAGIGDTPSLEDEAAGHVTQARMVSKSKDGTGSDDKKAKGADGKTKIATPRGAAPPGQKGQANATRIPAKTPPAPKTPPSSGEPPKSGDRSGYSSPGSPGTPGSRSRTPSLPTPPTREPKKVAVVRTPPKSPSSAKSRLQTAPVPMPDLKNVKSKIGSTENLKHQPGGGKVQIVYKPVDLSKVTSKCGSLGNIHHKPGGGQVEVKSEKLDFKDRVQSKIGSLDNITHVPGGGNKKIETHKLTFRENAKAKTDHGAEIVYKSPVVSGDTSPRHLSNVSSTGSIDMVDSPQLATLADEVSASLAKQGL

SEQ ID NO: 48 - DNA, 6670 bp, Artificial Sequence
  synthetic
tggcgaatgggacgcgccctgtagcggcgcattaagcgcggcgggtgtggtggttacgcgcagcgtgaccgctacacttgccagcgccctagcgcccgctcctttcgctttcttcccttcctttctcgccacgttcgccggctttccccgtcaagctctaaatcgggggctccctttagggttccgatttagtgctttacggcacctcgaccccaaaaaacttgattagggtgatggttcacgtagtgggccatcgccctgatagacggtttttcgccctttgacgttggagtccacgttctttaatagtggactcttgttccaaactggaacaacactcaaccctatctcggtctattcttttgatttataagggattttgccgatttcggcctattggttaaaaaatgagctgatttaacaaaaatttaacgcgaattttaacaaaatattaacgtttacaatttcaggtggcacttttcggggaaatgtgcgcggaacccctatttgtttatttttctaaatacattcaaatatgtatccgctcatgagacaataaccctgataaatgcttcaataatattgaaaaaggaagagtatgagtattcaacatttccgtgtcgcccttattcccttttttgcggcattttgccttcctgtttttgctcacccagaaacgctggtgaaagtaaaagatgctgaagatcagttgggtgcacgagtgggttacatcgaactggatctcaacagcggtaagatccttgagagttttcgccccgaagaacgttttccaatgatgagcacttttaaagttctgctatgtggcgcggtattatcccgtattgacgccgggcaagagcaactcggtcgccgcatacactattctcagaatgacttggttgagtactcaccagtcacagaaaagcatcttacggatggcatgacagtaagagaattatgcagtgctgccataaccatgagtgataacactgcggccaacttacttctgacaacgatcggaggaccgaaggagctaaccgcttttttgcacaacatgggggatcatgtaactcgccttgatcgttgggaaccggagctgaatgaagccataccaaacgacgagcgtgacaccacgatgcctgcagcaatggcaacaacgttgcgcaaactattaactggcgaactacttactctagcttcccggcaacaattaatagactggatggaggcggataaagttgcaggaccacttctgcgctcggcccttccggctggctggtttattgctgataaatctggagccggtgagcgtgggtctcgcggtatcattgcagcactggggccagatggtaagccctcccgtatcgtagttatctacacgacggggagtcaggcaactatggatgaacgaaatagacagatcgctgagataggtgcctcactgattaagcattggtaactgtcagaccaagtttactcatatatactttagattgatttaaaacttcatttttaatttaaaaggatctaggtgaagatcctttttgataatctcatgaccaaaatcccttaacgtgagttttcgttccactgagcgtcagaccccgtagaaaagatcaaaggatcttcttgagatcctttttttctgcgcgtaatctgctgcttgcaaacaaaaaaaccaccgctaccagcggtggtttgtttgccggatcaagagctaccaactctttttccgaaggtaactggcttcagcagagcgcagataccaaatactgtccttctagtgtagccgtagttaggccaccacttcaagaactctgtagcaccgcctacatacctcgctctgctaatcctgttaccagtggctgctgccagtggcgataagtcgtgtcttaccgggttggactcaagacgatagttaccggataaggcgcagcggtcgggctgaacggggggttcgtgcacacagcccagcttggagcgaacgacctacaccgaactgagatacctacagcgtgagctatgagaaagcgccacgcttcccgaagggagaaaggcggacaggtatccggtaagcggcagggtcggaacaggagagcgcacgagggagcttccagggggaaacgcctggtatctttatagtcctgtcgggtttcgccacctctgacttgagcgtcgatttttgtgatgctcgtcaggggggcggagcctatggaaaaacgccagcaacgcggcctttttacggttcctggccttttgctggccttttgctcacatgttctttcctgcgttatcccctgattctgtggataaccgtattaccgcctttgagtgagctgataccgctcgccgcagccgaacgaccgagcgcagcgagtcagtgagcgaggaagcggaagagcgcctgatgcggtattttctccttacgcatctgtgcggtatttcacaccgcatatatggtgcactctcagtacaatctgctctgatgccgcatagttaagccagtatacactccgctatcgctacgtgactgggtcatggctgcgccccgacacccgccaacacccgctgacgcgccctgacgggcttgtctgctcccggcatccgcttacagacaagctgtgaccgtctccgggagctgcatgtgtcagaggttttcaccgtcatcaccgaaacgcgcgaggcagctgcggtaaagctcatcagcgtggtcgtgaagcgattcacagatgtctgcctgttcatccgcgtccagctcgttgagtttctccagaagcgttaatgtctggcttctgataaagcgggccatgttaagggcggttttttcctgtttggtcactgatgcctccgtgtaagggggatttctgttcatgggggtaatgataccgatgaaacgagagaggatgctcacgatacgggttactgatgatgaacatgcccggttactggaacgttgtgagggtaaacaactggcggtatggatgcggcgggaccagagaaaaatcactcagggtcaatgccagcgcttcgttaatacagatgtaggtgttccacagggtagccagcagcatcctgcgatgcagatccggaacataatggtgcagggcgctgacttccgcgtttccagactttacgaaacacggaaaccgaagaccattcatgttgttgctcaggtcgcagacgttttgcagcagcagtcgcttcacgttcgctcgcgtatcggtgattcattctgctaaccagtaaggcaaccccgccagcctagccgggtcctcaacgacaggagcacgatcatgcgcacccgtggggccgccatgccggcgataatggcctgcttctcgccgaaacgtttggtggcgggaccagtgacgaaggcttgagcgagggcgtgcaagattccgaataccgcaagcgacaggccgatcatcgtcgcgctccagcgaaagcggtcctcgccgaaaatgacccagagcgctgccggcacctgtcctacgagttgcatgataaagaagacagtcataagtgcggcgacgatagtcatgccccgcgcccaccggaaggagctgactgggttgaaggctctcaagggcatcggtcgagatcccggtgcctaatgagtgagctaacttacattaattgcgttgcgctcactgcccgctttccagtcgggaaacctgtcgtgccagctgcattaatgaatcggccaacgcgcggggagaggcggtttgcgtattgggcgccagggtggtttttcttttcaccagtgagacgggcaacagctgattgcccttcaccgcctggccctgagagagttgcagcaagcggtccacgctggtttgccccagcaggcgaaaatcctgtttgatggtggttaacggcgggatataacatgagctgtcttcggtatcgtcgtatcccactaccgagatgtccgcaccaacgcgcagcccggactcggtaatggcgcgcattgcgcccagcgccatctgatcgttggcaaccagcatcgcagtgggaacgatgccctcattcagcatttgcatggtttgttgaaaaccggacatggcactccagtcgccttcccgttccgctatcggctgaatttgattgcgagtgagatatttatgccagccagccagacgcagacgcgccgagacagaacttaatgggcccgctaacagcgcgatttgctggtgacccaatgcgaccagatgctccacgcccagtcgcgtaccgtcttcatgggagaaaataatactgttgatgggtgtctggtcagagacatcaagaaataacgccggaacattagtgcaggcagcttccacagcaatggcatcctggtcatccagcggatagttaatgatcagcccactgacgcgttgcgcgagaagattgtgcaccgccgctttacaggcttcgacgccgcttcgttctaccatcgacaccaccacgctggcacccagttgatcggcgcgagatttaatcgccgcgacaatttgcgacggcgcgtgcagggccagactggaggtggcaacgccaatcagcaacgactgtttgcccgccagttgttgtgccacgcggttgggaatgtaattcagctccgccatcgccgcttccactttttcccgcgttttcgcagaaacgtggctggcctggttcaccacgcgggaaacggtctgataagagacaccggcatactctgcgacatcgtataacgttactggtttcacattcaccaccctgaattgactctcttccgggcgctatcatgccataccgcgaaaggttttgcgccattcgatggtgtccgggatctcgacgctctcccttatgcgactcctgcattaggaagcagcccagtagtaggttgaggccgttgagcaccgccgccgcaaggaatggtgcatgcaaggagatggcgcccaacagtcccccggccacggggcctgccaccatacccacgccgaaacaagcgctcatgagcccgaagtggcgagcccgatcttccccatcggtgatgtcggcgatataggcgccagcaaccgcacctgtggcgccggtgatgccggccacgatgcgtccggcgtagaggatcgagatcgatctcgatcccgcgaaattaatacgactcactataggggaattgtgagcggataacaattcccctctagaaataattttgtttaactttaagaaggagatatacatatgggctcaagccaccaccaccaccaccacagcagcggcgagaacttgtactttcaaggatccgcagaaccacgtcaagaatttgaggttatggaagatcacgcgggcacttacggtttgggtgatcgtaaagaccagggcggctataccatgcatcaagatcaagagggcgacaccgatgctggcttgaaagagtcgccgctgcagactccgaccgaggatggcagcgaagagccgggcagcgagactagcgatgcgaagtcgaccccgaccgccgaggcagaagaggcgggtatcggcgacactccgtccctggaagatgaggcagccggtcatgtcacgcaggcgcgtatggtgagcaagagcaaagatggtacgggtagcgacgacaagaaggcgaagggcgcagatggcaagaccaaaattgcgacgccgcgtggtgcggcaccgccaggccagaaaggtcaggcgaatgccacgcgcatcccggcaaagacgccaccggctccgaaaaccccgccttccagcggtgaaccgccgaaatccggtgaccgcagcggttatagctctccgggtagcccgggtaccccaggcagccgtagccgcaccccgagcctgccgaccccaccgacccgcgagccgaagaaagtggcggtggttcgtacgccgccaaaaagcccgagctctgccaagagccgtctgcaaaccgctcctgtgccgatgccggacctgaagaacgttaagtctaaaatcggtagcaccgaaaatctgaagcaccaacctggtggcggtaaggttcaaatcatcaacaaaaagctggacttgagcaatgtacaaagcaagtgtggtagcaaggacaatatcaaacacgtcccgggtggtggttccgtccagattgtgtacaaaccggtggacctgagcaaggttaccagcaaatgcggttccctgggtaacatccatcataaaccgggtggcggccaagttgaggtcaagagcgagaaactggacttcaaagaccgcgttcagtccaaaatcggttctctggacaacattacgcacgtgcctggtggtggcaacaagaagattgaaacccataaactgacgtttcgtgaaaatgcgaaggcgaaaaccgaccacggcgcagagattgtctacaaaagcccggtggtgagcggtgataccagcccgcgtcacctgtccaacgtcagcagcacgggcagcattgatatggtggatagcccgcagttggctacgctggccgatgaggttagcgcgagcctggcgaagcagggtctgtgactcgagcaccaccaccaccaccactgagatccggctgctaacaaagcccgaaaggaagctgagttggctgctgccaccgctgagcaataactagcataaccccttggggcctctaaacgggtcttgaggggttttttgctgaaaggaggaactatatccggat

SEQ ID NO: 49 - protein, 432 aa, Artificial Sequence
  synthetic
MGSSHHHHHHSSGENLYFQGSAEPRQEFEVMEDHAGTYGLGDRKDQGGYTMHQDQEGDTDAGLKESPLQTPTEDGSEEPGSETSDAKSTPTAEAEEAGIGDTPSLEDEAAGHVTQARMVSKSKDGTGSDDKKAKGADGKTKIATPRGAAPPGQKGQANATRIPAKTPPAPKTPPSSGEPPKSGDRSGYSSPGSPGTPGSRSRTPSLPTPPTREPKKVAVVRTPPKSPSSAKSRLQTAPVPMPDLKNVKSKIGSTENLKHQPGGGKVQIINKKLDLSNVQSKCGSKDNIKHVPGGGSVQIVYKPVDLSKVTSKCGSLGNIHHKPGGGQVEVKSEKLDFKDRVQSKIGSLDNITHVPGGGNKKIETHKLTFRENAKAKTDHGAEIVYKSPVVSGDTSPRHLSNVSSTGSIDMVDSPQLATLADEVSASLAKQGL

SEQ ID NO: 50 - protein, 413 aa, Artificial Sequence
  synthetic
GSAEPRQEFEVMEDHAGTYGLGDRKDQGGYTMHQDQEGDTDAGLKESPLQTPTEDGSEEPGSETSDAKSTPTAEAEEAGIGDTPSLEDEAAGHVTQARMVSKSKDGTGSDDKKAKGADGKTKIATPRGAAPPGQKGQANATRIPAKTPPAPKTPPSSGEPPKSGDRSGYSSPGSPGTPGSRSRTPSLPTPPTREPKKVAVVRTPPKSPSSAKSRLQTAPVPMPDLKNVKSKIGSTENLKHQPGGGKVQIINKKLDLSNVQSKCGSKDNIKHVPGGGSVQIVYKPVDLSKVTSKCGSLGNIHHKPGGGQVEVKSEKLDFKDRVQSKIGSLDNITHVPGGGNKKIETHKLTFRENAKAKTDHGAEIVYKSPVVSGDTSPRHLSNVSSTGSIDMVDSPQLATLADEVSASLAKQGL

SEQ ID NO: 51 - DNA, 6016 bp, Artificial Sequence
  synthetic
gctgcttcgcgatgtacgggccagatatacgcgttttgagatttctgtcgccgactaaattcatgtcgcgcgatagtggtgtttatcgccgatagagatggcgatattggaaaaatcggcggccgccgatatttgaaaatatggcatattgaaaatgtcgccgatgtgagtttctgtgtaactgacatcgccatttttccaaaagtgatttttgggcatacgcggtatctggcgatagcgcttatatcgtttacgggggatggcgatagacgactttggtgacttgggcgattctgtgtgtcgcaaatatcgcagtttcgatataggtgacagacgatatgaggctatatcgccgatagaggcgacatcaagctggcacatggccaatgcatatcgatctatacattgaatcaatattggccattagccatattattcattggttatatagcataaatcaatattggctattggccattgcatacgttgtatccatatcataatatgtacatttatattggctcatgtccaacattaccgccatgttgacattgattattgactagttattaatagtaatcaattacggggtcattagttcatagcccatatatggagttccgcgttacataacttacggtaaatggcccgcctggctgaccgcccaacgacccccgcccattgacgtcaataatgacgtatgttcccatagtaacgccaatagggactttccattgacgtcaatgggtggagtatttacggtaaactgcccacttggcagtacatcaagtgtatcatatgccaagtacgccccctattgacgtcaatgacggtaaatggcccgcctggcattatgcccagtacatgaccttatgggactttcctacttggcagtacatctacgtattagtcatcgctattacaatggtgatgcggttttggcagtacatcaatgggcgtggatagcggtttgactcacggggatttccaagtctccaccccattgacgtcaatgggagtttgttttggcaccaaaatcaacgggactttccaaaatgtcgtaacaactccgccccattgacgcaaatgggcggtaggcgtgtacggtgggaggtctatataagcagaactcgtttagtgaaccgtcagatcgcctggagacgccatccacgctgttttgacctccatagaagacaccgggaccgatccagcctccgcggccgggaacggtgcattggaacgcggattccccgtgccaagagtgacgtaagtaccgcctatagagtctataggcccaccccattggcttcttatgcatgctatactgtttttggcttggggtctatacacccccgcttcctcatgttataggtgatggtatagcttagcctataggtgtgggttattgaccattattgaccactcccctattggtgacgatactttccattactaatccataacatggctctttgccacaactctctttattggctatatgccaatacactgtccttcagagactgacacggactctgtatttttacaggatggggtctcatttattatttacaaattcacatatacaacaccaccgtccccagtgcccgcagtttttattaaacataacgtgggatctccacgcgaatctagggtacgtgttacggacatgggctattctcaggtagcggcggagcttctacatccgagccctgctcccatgcctccagcgaatcatggtcgctcggcagctccttgctcctaacagtggaggccagacttaggcacagcacgatgcccaccaccaccagtgtgccgcacaaggccgtggcggtagggtatgtgtctgaaaatgaactaggggagcgggcttgcaccgctgacgcatttggaagacttaaggcagcggcagaagaagatgcaggcaactgagttgttgtgttctgataagagtcagaggtaactcccgttgcggtgctgttaacggtggagggcagtgtagtctgagcagtactcgttgctgccgcacgcgccaccagacataatagctgacagactaacagactgttcctttcaatgggtcttttatgcagtcaccgtccttgacacgaagcttgccaccatgggctcaagccaccatcaccaccaccatcatcaccaccacagcagcggcgagaacttgtactttcaaggatccgctgagccccgccaggagttcgaagtgatggaagatcacgctgggacgtacgggttgggggacaggaaagatcaggggggctacaccatgcaccaagaccaagagggtgacacggacgctggcctgaaagaatctcccctgcagacccccactgaggacggatctgaggaaccgggctctgaaacctctgatgctaagagcactccaacagcggaagatgtgacagcacccttagtggatgagggagctcccggcaagcaggctgccgcgcagccccacacggagatcccagaaggaaccacagctgaagaagcaggcattggagacacccccagcctggaagacgaagctgctggtcacgtgacccaagctcgcatggtcagtaaaagcaaagacgggactggaagcgatgacaaaaaagccaagggggctgatggtaaaacgaagatcgccacaccgcggggagcagcccctccaggccagaagggccaggccaacgccaccaggattccagcaaaaaccccgcccgctccaaagacaccacccagctctggtgaacctccaaaatcaggggatcgcagcggctacagcagccccggctccccaggcactcccggcagccgctcccgcaccccgtcccttccaaccccacccacccgggagcccaagaaggtggcagtggtccgtactccacccaagtcgccgtcttccgccaagagccgcctgcagacagcccccgtgcccatgccagacctgaagaatgtcaagtccaagatcggctccactgagaacctgaagcaccagccgggaggcgggaaggtgcagataattaataagaagctggatcttagcaacgtccagtccaagtgtggctcaaaggataatatcaaacacgtcccgggaggcggcagtgtgcaaatagtctacaaaccagttgacctgagcaaggtgacctccaagtgtggctcattaggcaacatccatcataaaccaggaggtggccaggtggaagtaaaatctgagaagctagacttcaaggacagagtccagtcgaagattgggtccctggacaatatcacccacgtccctggcggaggaaataaaaagattgaaacccacaagctgaccttccgcgagaacgccaaagccaagacagaccacggggcggagatcgtgtacaagtcgccagtggtgtctggggacacgtctccacggcatctcagcaatgtctcctccaccggcagcatcgacatggtagactcgccccagctcgccacgctagctgacgaggtgtctgcctccctggccaagcagggtttgtgactcgaggagaacttgtacttccagggaagtggtggcagtcatcaccatcaccatcaccatcaccatcactgagaattcattgatcataatcagccataccacatttgtagaggttttacttgctttaaaaaacctcccacacctccccctgaacctgaaacataaaatgaatgcaattgttgttgttaacttgtttattgcagcttataatggttacaaataaagcaatagcatcacaaatttcacaaataaagcatttttttcactgcattctagttgtggtttgtccaaactcatcaatgtatcttatcatgtctgaatcctctacgccggacgcatcgtggccggcatcaccggcgccacaggtgcggttgctggcgcctatatcgccgacatcaccgatggggaagatcgggctcgccacttcgggctcatgagcgcttgtttcggcgtgggtatggtggcaggccccgtggccgggggactgttgggcgccatctccttgcatgcaccattccttgcggcggcggtgctcaacggcctcaacctactactgggctgcttcctaatgcaggagtcgcataagggagagcgtcgactggggcgccctctggtaaggttgggaagccctgcaaagtaaactggatggctttctcgccgccaagcatctgatggcgcaggggatcaagctctgatcaagagacaggatgaggatcgtttcgcatgattgaacaagatggattgcacgcaggttctccggccgcttgggtggagaggctattcggctatgactgggcacaacagacaatcggctgctctgatgccgccgtgttccggctgtcagcgcaggggcgcccggttctttttgtcaagaccgacctgtccggtgccctgaatgaactgcaagacgaggcagcgcggctatcgtggctggccacgacgggcgttccttgcgcagcagtgctcgacgttgtcactgaagcgggaagggactggctgctattgggcgaagtgccggggcaggatctcctgtcatctcaccttgctcctgccgagaaagtatccatcatggctgatgcaatgcggcggctgcatacgcttgatccggctacctgcccattcgaccaccaagcgaaacatcgcatcgagcgagcacgtactcggatggaagccggtcttgtcgatcaggatgatctggacgaagagcatcaggggctcgcgccagccgaactgttcgccaggctcaaggcgagcatgcccgacggcgaggatctcgtcgtgacccacggcgatgcctgcttgccgaatatcatggtggaaaatggccgcttttctggattcatcgactgtggccggctgggtgtggcggaccgctatcaggacatagcgttggctacccgtgatattgctgaagagcttggcggcgaatgggctgaccgcttcctcgtgctttacggtatcgccgctcccgattcgcagcgcatcgccttctatcgccttcttgacgagttcttctgaattattaacgcttacaatttcctgatgcggtattttctccttacgcatctgtgcggtatttcacaccgcatcaggtggcacttttcggggaaatgtgcgcggaacccctatttgtttatttttctaaatacattcaaatatgtatccgctcatgagacaataaccctgataaatgcttcaataatagcacgtgctaaaacttcatttttaatttaaaaggatctaggtgaagatcctttttgataatctcatgaccaaaatcccttaacgtgagttttcgttccactgagcgtcagaccccgtagaaaagatcaaaggatcttcttgagatcctttttttctgcgcgtaatctgctgcttgcaaacaaaaaaaccaccgctaccagcggtggtttgtttgccggatcaagagctaccaactctttttccgaaggtaactggcttcagcagagcgcagataccaaatactgttcttctagtgtagccgtagttaggccaccacttcaagaactctgtagcaccgcctacatacctcgctctgctaatcctgttaccagtggctgctgccagtggcgataagtcgtgtcttaccgggttggactcaagacgatagttaccggataaggcgcagcggtcgggctgaacggggggttcgtgcacacagcccagcttggagcgaacgacctacaccgaactgagatacctacagcgtgagctatgagaaagcgccacgcttcccgaagggagaaaggcggacaggtatccggtaagcggcagggtcggaacaggagagcgcacgagggagcttccagggggaaacgcctggtatctttatagtcctgtcgggtttcgccacctctgacttgagcgtcgatttttgtgatgctcgtcaggggggcggagcctatggaaaaacgccagcaacgcggcctttttacggttcctggccttttgctggccttttgctcacatgttctt

SEQ ID NO: 52 - protein, 465 aa, Artificial Sequence
  synthetic
MGSSHHHHHHHHHHSSGENLYFQGSAEPRQEFEVMEDHAGTYGLGDRKDQGGYTMHQDQEGDTDAGLKESPLQTPTEDGSEEPGSETSDAKSTPTAEDVTAPLVDEGAPGKQAAAQPHTEIPEGTTAEEAGIGDTPSLEDEAAGHVTQARMVSKSKDGTGSDDKKAKGADGKTKIATPRGAAPPGQKGQANATRIPAKTPPAPKTPPSSGEPPKSGDRSGYSSPGSPGTPGSRSRTPSLPTPPTREPKKVAVVRTPPKSPSSAKSRLQTAPVPMPDLKNVKSKIGSTENLKHQPGGGKVQIINKKLDLSNVQSKCGSKDNIKHVPGGGSVQIVYKPVDLSKVTSKCGSLGNIHHKPGGGQVEVKSEKLDFKDRVQSKIGSLDNITHVPGGGNKKIETHKLTFRENAKAKTDHGAEIVYKSPVVSGDTSPRHLSNVSSTGSIDMVDSPQLATLADEVSASLAKQGL

SEQ ID NO: 53 - protein, 442 aa, Artificial Sequence; identical to SEQ ID NO: 41
  synthetic

SEQ ID NO: 54 - protein, 448 aa, Artificial Sequence
  humanized
EVQLQESGPGLVKPSETLSLTCTVSGFSLTSNDIAWIRQPPGKGLEWMGTIWTDGSTNYNAAVQSRVTISVDTSKNQFSLKLSSVTAADTAVYYCARHRLYYGAFDYWGQGTMVTVSSASTKGPSVFPLAPSSKSTSGGTAALGCLVKDYFPEPVTVSWNSGALTSGVHTFPAVLQSSGLYSLSSVVTVPSSSLGTQTYICNVNHKPSNTKVDKKVEPKSCDKTHTCPPCPAPELLGGPSVFLFPPKPKDTLMISRTPEVTCVVVDVSHEDPEVKFNWYVDGVEVHNAKTKPREEQYNSTYRVVSVLTVLHQDWLNGKEYKCKVSNKALPAPIEKTISKAKGQPREPQVYTLPPSRDELTKNQVSLTCLVKGFYPSDIAVEWESNGQPENNYKTTPPVLDSDGSFFLYSKLTVDKSRWQQGNVFSCSVMHEALHNHYTQKSLSLSPGK

SEQ ID NO: 55 - protein, 448 aa, Artificial Sequence
  humanized
EVQLQESGPGLVKPSETLSLTCTVSGFSLTSNDIAWIRQPPGKGLEWMGTIWTDGSTNYNTAVQSRVTISVDTSKNQFSLKLSSVTAADTAVYYCARHRLYYGAFDYWGQGTMVTVSSASTKGPSVFPLAPSSKSTSGGTAALGCLVKDYFPEPVTVSWNSGALTSGVHTFPAVLQSSGLYSLSSVVTVPSSSLGTQTYICNVNHKPSNTKVDKKVEPKSCDKTHTCPPCPAPELLGGPSVFLFPPKPKDTLMISRTPEVTCVVVDVSHEDPEVKFNWYVDGVEVHNAKTKPREEQYNSTYRVVSVLTVLHQDWLNGKEYKCKVSNKALPAPIEKTISKAKGQPREPQVYTLPPSRDELTKNQVSLTCLVKGFYPSDIAVEWESNGQPENNYKTTPPVLDSDGSFFLYSKLTVDKSRWQQGNVFSCSVMHEALHNHYTQKSLSLSPGK

SEQ ID NO: 56 - DNA, 1344 bp, Artificial Sequence
  humanized
gaggtgcagctgcaggaatccggtcccggcctcgtgaagccttcagaaaccctgtcgctcacatgcactgtgtccgggttctccctgacctctaacgacatcgcctggattcggcagccgccaggaaagggactggagtggatgggcaccatttggaccgacgggtcaaccaactacaatgccgcggtgcaatccagagtgaccatcagcgtggacacgtccaagaaccagttctcgctgaaattgagctccgtgactgccgctgatactgccgtgtattactgtgcccggcaccgcctttactacggcgcatttgactactggggacagggaaccatggtcactgtctcgagtgcctccaccaagggcccctccgtgttcccgctcgctccatcatcgaagtctaccagcggaggcactgcggctctcggttgcctcgtgaaggactacttcccggagccggtgaccgtgtcgtggaacagcggagccctgaccagcggggtgcacacctttccggccgtcttgcagtcaagcggcctttactccctgtcatcagtggtgactgtcccgtccagctcattgggaacccaaacctacatctgcaatgtgaatcacaaacctagcaacaccaaggttgacaagaaagtcgagcccaaatcgtgtgacaagactcacacttgtccgccgtgcccggcacccgaactgctgggaggtcccagcgtctttctgttccctccaaagccgaaagacacgctgatgatctcccgcaccccggaggtcacttgcgtggtcgtggacgtgtcacatgaggacccagaggtgaagttcaattggtacgtggatggcgtcgaagtccacaatgccaaaactaagcccagagaagaacagtacaattcgacctaccgcgtcgtgtccgtgctcacggtgttgcatcaggattggctgaacgggaaggaatacaagtgcaaagtgtccaacaaggcgctgccggcaccgatcgagaaaactatctccaaagcgaagggacagcctagggaacctcaagtctacacgctgccaccatcacgggatgaactgactaagaatcaagtctcactgacttgtctggtgaaggggttttaccctagcgacattgccgtggagtgggaatccaacggccagccagagaacaactacaagactacccctccagtgctcgactcggatggatcgttcttcctttactcgaagctcaccgtggataagtcccggtggcagcagggaaacgtgttctcctgctcggtgatgcatgaagccctccataaccactatacccaaaagtcgctgtccctgtcgccgggaaag

SEQ ID NO: 57 - DNA, 1344 bp, Artificial Sequence
  humanized
gaggtgcaactgcaggaatccggtcccggcctcgtgaagccttcagaaaccctgtcgctcacatgcactgtgtccgggttctccctgacctctaacgacatcgcctggattcggcagccgccaggaaagggactggagtggatgggcaccatttggaccgacgggtcaaccaactacaataccgcggtgcaatccagagtgaccatcagcgtggacacgtccaagaaccagttctcgctgaaattgagctccgtgactgccgctgatactgccgtgtattactgtgcccggcaccgcctttactacggcgcatttgactactggggacagggaaccatggtcactgtctcgagtgcctccaccaagggcccctccgtgttcccgctcgctccatcatcgaagtctaccagcggaggcactgcggctctcggttgcctcgtgaaggactacttcccggagccggtgaccgtgtcgtggaacagcggagccctgaccagcggggtgcacacctttccggccgtcttgcagtcaagcggcctttactccctgtcatcagtggtgactgtcccgtccagctcattgggaacccaaacctacatctgcaatgtgaatcacaaacctagcaacaccaaggttgacaagaaagtcgagcccaaatcgtgtgacaagactcacacttgtccgccgtgcccggcacccgaactgctgggaggtcccagcgtctttctgttccctccaaagccgaaagacacgctgatgatctcccgcaccccggaggtcacttgcgtggtcgtggacgtgtcacatgaggacccagaggtgaagttcaattggtacgtggatggcgtcgaagtccacaatgccaaaactaagcccagagaagaacagtacaattcgacctaccgcgtcgtgtccgtgctcacggtgttgcatcaggattggctgaacgggaaggaatacaagtgcaaagtgtccaacaaggcgctgccggcaccgatcgagaaaactatctccaaagcgaagggacagcctagggaacctcaagtctacacgctgccaccatcacgggatgaactgactaagaatcaagtctcactgacttgtctggtgaaggggttttaccctagcgacattgccgtggagtgggaatccaacggccagccagagaacaactacaagactacccctccagtgctcgactcggatggatcgttcttcctttactcgaagctcaccgtggataagtcccggtggcagcagggaaacgtgttctcctgctcggtgatgcatgaagccctccataaccactatacccaaaagtcgctgtccctgtcgccgggaaag